European Patent Application EP 4 793 366 A1, published August 19, 2026. Title: Method for degrading 5' terminal adenylated single-stranded DNA, method for ligation to nucleic acid, method for preparing NGS library, NGS library preparation kit, and 3' adapter for nucleic acid library preparation. Applicant: ARKRAY, Inc. The sequence listing filed with the application follows.

SEQUENCE LISTING (14 sequences)

SEQ ID NO: 1 - RNA, 26 nt, synthetic construct
  source 1..26: mol_type = other RNA
gttcagagttctacagtccgacgatc

SEQ ID NO: 2 - DNA, 65 bp, synthetic construct
  source 1..65: mol_type = other DNA
gtgactggagttcagacgtgtgctcttccgatctnnnnnnnnnnnnattgatggtgcctacagtt

SEQ ID NO: 3 - DNA, 55 bp, synthetic construct
  source 1..55: mol_type = other DNA
caagcagaagacggcatacgagatcgtgatgctccaccgataaatattagcccgt

SEQ ID NO: 4 - DNA, 50 bp, synthetic construct
  source 1..50: mol_type = other DNA
aatgatacggcgaccaccgagatctacacgttcagagttctacagtccga

SEQ ID NO: 5 - DNA, 61 bp, synthetic construct
  source 1..61: mol_type = other DNA
gtgactggagttcagacgtgtgctcttccgatctnnnnnnnnnnnnattgatggtgcctac

SEQ ID NO: 6 - DNA, 19 bp, synthetic construct
  source 1..19: mol_type = other DNA
  modified_base 19: mod_base = OTHER; note = modified by dideoxycytidine
  modified_base 1: mod_base = OTHER; note = modified by adenylic acid
nnnngtaggcaccatcaat

SEQ ID NO: 7 - DNA, 19 bp, synthetic construct
  source 1..19: mol_type = other DNA
  modified_base 19: mod_base = OTHER; note = modified by dideoxycytidine
  modified_base 1: mod_base = OTHER; note = modified by adenylic acid
gtatgtaggcaccatcaat

SEQ ID NO: 8 - DNA, 19 bp, synthetic construct
  source 1..19: mol_type = other DNA
  modified_base 19: mod_base = OTHER; note = modified by dideoxycytidine
  modified_base 1: mod_base = OTHER; note = modified by adenylic acid
gacagtaggcaccatcaat

SEQ ID NO: 9 - DNA, 19 bp, synthetic construct
  source 1..19: mol_type = other DNA
  modified_base 1: mod_base = OTHER; note = modified by adenylic acid
  modified_base 19: mod_base = OTHER; note = modified by dideoxycytidine
aactgtaggcaccatcaat

SEQ ID NO: 10 - DNA, 19 bp, synthetic construct
  source 1..19: mol_type = other DNA
  modified_base 19: mod_base = OTHER; note = modified by dideoxycytidine
  modified_base 1: mod_base = OTHER; note = modified by adenylic acid
aacagtaggcaccatcaat

SEQ ID NO: 11 - DNA, 19 bp, synthetic construct
  source 1..19: mol_type = other DNA
  modified_base 19: mod_base = OTHER; note = modified by dideoxycytidine
  modified_base 1: mod_base = OTHER; note = modified by adenylic acid
tccagtaggcaccatcaat

SEQ ID NO: 12 - DNA, 19 bp, synthetic construct
  source 1..19: mol_type = other DNA
  modified_base 19: mod_base = OTHER; note = modified by dideoxycytidine
  modified_base 1: mod_base = OTHER; note = modified by adenylic acid
aacggtaggcaccatcaat

SEQ ID NO: 13 - DNA, 19 bp, synthetic construct
  source 1..19: mol_type = other DNA
  modified_base 19: mod_base = OTHER; note = modified by dideoxycytidine
  modified_base 1: mod_base = OTHER; note = modified by adenylic acid
cccagtaggcaccatcaat

SEQ ID NO: 14 - DNA, 19 bp, synthetic construct
  source 1..19: mol_type = other DNA
  modified_base 19: mod_base = OTHER; note = modified by dideoxycytidine
  modified_base 1: mod_base = OTHER; note = modified by adenylic acid
aggagtaggcaccatcaat